European Patent Application EP 4 400 510 A2, published July 17, 2024. Title: IMPROVED VACCINES AND METHODS FOR USING THE SAME. Applicant: The Trustees of the University of Pennsylvania. The sequence listing filed with the application follows.

SEQUENCE LISTING (44 sequences)

SEQ ID NO: 1 - DNA, 2142 bp, synthetic construct
  misc_feature 1..2142: note = Subtype A consensus Envelope DNA sequence construct
  source 1..2142: mol_type = other DNA
ggatccatggactggacctggattctgttcctggtggccgccgccaccagagtgcacagcagagtgatgggcatccagcggaattgccagcacctgtggagatggggcaccatgatcctgggcatgatcatcatctgctctgccgccgagaacctgtgggtgaccgtgtactacggcgtgcctgtgtggaaggacgccgagaccaccctgttctgcgccagcgacgccaaggcctacgataccgaagtgcacaatgtgtgggccacccacgcctgcgtgcctaccgatcccaacccccaggagatcaacctggagaacgtgaccgaggagttcaacatgtggaagaacaacatggtggagcagatgcacaccgacatcatcagcctgtgggaccagagcctgaagccttgcgtgaagctgacccctctgtgcgtgaccctgaactgcagcaacgtgaacgtgaccaccaacatcatgaagggcgagatcaagaactgcagcttcaacatgaccaccgagctgcgggacaagaagcagaaagtgtacagcctgttctacaagctggacgtggtgcagatcaacaagagcaacagcagcagccagtaccggctgatcaactgcaacaccagcgccatcacccaggcctgccccaaagtgagcttcgagcccatccccatccactactgcgcccctgccggcttcgccatcctgaagtgcaaggacaaggagtttaacggcaccggcccctgcaagaatgtgagcaccgtgcagtgcacccacggcatcaagcccgtggtgtccacccagctgctgctgaacggcagcctggccgaggaggaagtgatgatccggagcgagaacatcaccaacaacgccaagaacatcatcgtgcagctgaccaagcccgtgaagatcaattgcacccggcccaacaacaacacccggaagagcatcagaatcggccctggccaggccttctacgccaccggcgacatcatcggcgatatcaggcaggcccactgcaatgtgagccggaccgagtggaacgagaccctgcagaaagtggccaagcagctgcggaagtacttcaacaacaagaccatcatcttcaccaacagcagcggcggcagactgagaatcaccacccacagcttcaattgtggcggcgagttcttctactgcaatacctccggcctgttcaacagcacctggaacggcaacggcaccaagaagaagaacagcaccgagagcaacgacaccatcaccctgccctgccggatcaagcagatcatcaatatgtggcagagggtgggccaggccatgtacgcccctcccatccagggcgtgatcagatgcgagagcaacatcaccggcctgctgctgaccagagatggcggcgacaacaacagcaagaacgagaccttcagacctggcggcggagacatgagggacaactggcggagcgagctgtacaagtacaaagtggtgaagatcgagcccctgggcgtggcccccaccaaggccaagagaagagtggtggagcgggagaagagagctgtgggcatcggcgccgtgttcctgggcttcctgggagccgccggaagcaccatgggagccgccagcatcaccctgaccgtgcaggccagacagctgctgagcggcattgtgcagcagcagagcaacctgctgagagccatcgaggcccagcagcacctgctgaagctgacagtgtggggcatcaaacagctgcaggcccgcgtgctggccgtggagagatacctgaaggaccagcagctgctgggcatctggggctgcagcggcaagctgatctgcaccaccaacgtgccctggaatagcagctggagcaacaagagccagagcgagatctgggacaacatgacctggctgcagtgggacaaggagatcagcaactacaccgatatcatctacaacctgatcgaggagagccagaaccagcaggagaagaacgagcaggatctgctggccctggacaagtgggccaacctgtggaactggttcgacatcagcaactggctgtggtacatcaagatcttcatcatgattgtgggcggcctgatcggcctgagaatcgtgttcgccgtgctgtctgtgtgactcgag

SEQ ID NO: 2 - protein, 709 aa, synthetic construct
  REGION 1..709: note = Subtype A consensus Envelope protein sequence construct
MDWTWILFLVAAATRVHSRVMGIQRNCQHLWRWGTMILGMIIICSAAENLWVTVYYGVPVWKDAETTLFCASDAKAYDTEVHNVWATHACVPTDPNPQEINLENVTEEFNMWKNNMVEQMHTDIISLWDQSLKPCVKLTPLCVTLNCSNVNVTTNIMKGEIKNCSFNMTTELRDKKQKVYSLFYKLDVVQINKSNSSSQYRLINCNTSAITQACPKVSFEPIPIHYCAPAGFAILKCKDKEFNGTGPCKNVSTVQCTHGIKPVVSTQLLLNGSLAEEEVMIRSENITNNAKNIIVQLTKPVKINCTRPNNNTRKSIRIGPGQAFYATGDIIGDIRQAHCNVSRTEWNETLQKVAKQLRKYFNNKTIIFTNSSGGRLRITTHSFNCGGEFFYCNTSGLFNSTWNGNGTKKKNSTESNDTITLPCRIKQIINMWQRVGQAMYAPPIQGVIRCESNITGLLLTRDGGDNNSKNETFRPGGGDMRDNWRSELYKYKVVKIEPLGVAPTKAKRRVVEREKRAVGIGAVFLGFLGAAGSTMGAASITLTVQARQLLSGIVQQQSNLLRAIEAQQHLLKLTVWGIKQLQARVLAVERYLKDQQLLGIWGCSGKLICTTNVPWNSSWSNKSQSEIWDNMTWLQWDKEISNYTDIIYNLIEESQNQQEKNEQDLLALDKWANLWNWFDISNWLWYIKIFIMIVGGLIGLRIVFAVLSV

SEQ ID NO: 3 - DNA, 2734 bp, synthetic construct
  misc_feature 1..2734: note = Subtype B consensus Envelope DNA sequence construct
  source 1..2734: mol_type = other DNA
ggatccgccaccatggactggacctggattctgttcctggtggccgccgccaccagagtgcacagcagagtgaagggcatccggaagaactaccagcacctgtggagatggggcaccatgctgctgggcatgctgatgatctgttctgccgccgagaagctgtgggtgaccgtgtactacggcgtgcctgtgtggaaggaggccaccaccaccctgttctgcgccagcgacgccaaggcctacgataccgaagtgcacaatgtgtgggccacccacgcctgcgtgcctaccgatcccaaccctcaggaagtggtgctggagaacgtgaccgagaacttcaacatgtggaagaacaacatggtggagcagatgcacgaggacatcatcagcctgtgggaccagagcctgaagccttgcgtgaagctgacccctctgtgcgtgaccctgaactgcaccgacctgagcggcgagaagatggagaagggcgagatcaagaactgcagcttcaacatcaccacctccatccgggacaaagtgcagaaggagtacgccctgttctacaagctggacgtggtgcccatcgacaacgacaacaccagctaccggctgatcagctgcaacaccagcgtgatcacccaggcctgccccaaagtgagcttcgagcccatccccatccactactgcgcccctgccggcttcgccatcctgaagtgcaacgacaagaagttcaacggcaccggcccttgcaccaatgtgagcaccgtgcagtgcacccacggcatcagacccgtggtgtccacccagctgctgctgaacggcagcctggccgaggaagaagtggtgatccggagcgagaatttcaccaacaacgccaagaccatcatcgtgcagctgaacgagagcgtggagatcaactgcacccggcccaacaacaatacccggaagagcatccacatcggccctggccaggccttctacaccaccggcgagatcatcggcgatatcaggcaggcccactgcaatatcagccgggccaagtggaacaacaccctgaagcagatcgtgaagaagctgcgggagcagttcggcaacaagaccatcgtgttcaaccagagcagcggcggcagacctagaatcgtgatgcacagcttcaactgtggcggcgagttcttctactgcaacacaacccagctgttcaacagcacctggaacgtgaacgggacctggaacaacaacaccgagggcaacgacaccatcaccctgccctgccggatcaagcagatcatcaatatgtggcaggaggtgggcaaggccatgtacgcccctcccatcagaggccagatccggtgcagcagcaatatcaccggcctgctgctgaccagagatggcggcaacaataacaccaacgagaccgagatctttagacctggcggcggagacatgagggacaactggcggagcgagctgtacaagtacaaagtggtgaagatcgagcccctgggcgtggcccccaccaaggccaagagaagagtggtgcagcgggagaagagagctgtgggcatcggcgccatgtttctgggctttctgggagccgccggaagcaccatgggagccgccagcatgaccctgaccgtgcaggccagacagctgctgagcggcatcgtgcagcagcagaacaacctgctgagagccatcgaggcccagcagcacctgctgcagctgacagtgtggggcatcaagcagctgcaggcccgcgtgctggccgtggagagatacctgaaggaccagcagctgctgggaatctggggctgcagcggcaagctgatctgcaccaccaccgtgccctggaacgccagctggagcaacaagagcctggacgagatctgggacaacatgacctggatggagtgggagcgggagatcgacaactacaccagcctgatctacaccctgatcgaggagagccagaaccagcaggagaagaacgagcaggagctgctggagctggacaagtgggccagcctgtggaactggttcgacatcaccaactggctgtggtacatcaagatcttcatcatgattgtgggcggcctgatcggcctgagaatcgtgttcgccgtgctgagcatctacccctacgacgtgcccgattacgcctgagaattcgtaagtaagtgtcatatgggagagctcgactagactggacagccaatgacgggtaagagagtgacatttctcactaacctaagacaggagggccgtcaaagctactgcctaatccaatgacgggtaatagtgacaagaaatgtatcactccaacctaagacaggcgcagcctccgagggatgtgtcttttgttttttataattaaaaagggtgacatgtccggagccgtgctgcccggatgatgtcttggcctctgtttgctaccggtatcgatgttaacgtcgaccccgggctcgaggtaagtaagtgtcatatgggagagctcgactagactggacagccaatgacgggtaagagagtgacatttctcactaacctaagacaggagggccgtcaaagctactgcctaatccaatgacgggtaatagtgacaagaaatgtatcactccaacctaagacaggcgcagcctccgagggatgtgtcttttgttttttataattaaaaagggtgacatgtccggagccgtgctgcccggatgatgtcttggcctctgtttgctgcggccgc

SEQ ID NO: 4 - protein, 715 aa, synthetic construct
  REGION 1..715: note = Subtype B consensus Envelope protein sequence construct
MDWTWILFLVAAATRVHSRVKGIRKNYQHLWRWGTMLLGMLMICSAAEKLWVTVYYGVPVWKEATTTLFCASDAKAYDTEVHNVWATHACVPTDPNPQEVVLENVTENFNMWKNNMVEQMHEDIISLWDQSLKPCVKLTPLCVTLNCTDLSGEKMEKGEIKNCSFNITTSIRDKVQKEYALFYKLDVVPIDNDNTSYRLISCNTSVITQACPKVSFEPIPIHYCAPAGFAILKCNDKKFNGTGPCTNVSTVQCTHGIRPVVSTQLLLNGSLAEEEVVIRSENFTNNAKTIIVQLNESVEINCTRPNNNTRKSIHIGPGQAFYTTGEIIGDIRQAHCNISRAKWNNTLKQIVKKLREQFGNKTIVFNQSSGGRPRIVMHSFNCGGEFFYCNTTQLFNSTWNVNGTWNNNTEGNDTITLPCRIKQIINMWQEVGKAMYAPPIRGQIRCSSNITGLLLTRDGGNNNTNETEIFRPGGGDMRDNWRSELYKYKVVKIEPLGVAPTKAKRRVVQREKRAVGIGAMFLGFLGAAGSTMGAASMTLTVQARQLLSGIVQQQNNLLRAIEAQQHLLQLTVWGIKQLQARVLAVERYLKDQQLLGIWGCSGKLICTTTVPWNASWSNKSLDEIWDNMTWMEWEREIDNYTSLIYTLIEESQNQQEKNEQELLELDKWASLWNWFDITNWLWYIKIFIMIVGGLIGLRIVFAVLSIYPYDVPDYA

SEQ ID NO: 5 - DNA, 2140 bp, synthetic construct
  misc_feature 1..2140: note = Subtype C consensus Envelope DNA sequence construct
  source 1..2140: mol_type = other DNA
ggatccgccaccatggattggacctggattctgttcctggtggccgccgccacaagagtgcacagcagagtgcggggcatcctgagaaattgccagcagtggtggatctggggcattctggggttctggatgctgatgatctgcaacgtgatgggcaacctgtgggtgaccgtgtactacggcgtgcctgtgtggaaggaggccaagaccaccctgttctgtgccagcgatgccaaggcctacgagaccgaggtgcacaatgtgtgggccacccacgcctgtgtgcccaccgatcccaaccctcaggagatggtgctggagaacgtgaccgagaacttcaacatgtggaagaacgacatggtggaccagatgcacgaggacatcatcagcctgtgggaccagagcctgaagccttgcgtgaagctgacccctctgtgcgtgaccctgaactgccggaacaacgtgaacaacaacaacaccatgaaggaggagatcaagaactgcagcttcaacatcaccaccgagctgcgggacaagaagcagaaggtgtacgccctgttctaccggctggacatcgtgcccctgaacgagaagaacaacagcaacgactaccggctgatcaactgcaacaccagcgccatcacccaggcctgtcccaaggtgtccttcgaccccatccccatccactattgtgcccctgccggctacgccatcctgaagtgcaacaacaagaccttcaacggcaccggcccctgcaataatgtgagcaccgtgcagtgtacccacggcatcaagcctgtggtgtccacccagctgctgctgaatggcagcctggccgaggaggagattatcatccggagcgagaacctgaccaacaacgccaagaccatcattgtgcacctgaatgagagcgtggagatcgtgtgtacccggcccaacaacaatacccggaagagcatcagaatcggccctggccagaccttttacgccaccggcgacatcatcggcgatatcaggcaggcccactgcaatatcagcgaggagaagtggaacaagaccctgcagcgggtgtccgagaagctgaaggagcacttccccaataagaccatcaagttcgcccctagcagcggcggcagactggagatcaccacccacagcttcaactgcaggggcgagttcttctactgcaataccagcaagctgttcaacagcacctacatgcccaacagcaccaacaataccaacaccaccatcaccctgccctgccggatcaagcagatcatcaatatgtggcaggaagtgggcagagccatgtacgcccctcccatcgagggcaacatcacctgcaagtccaacatcaccggcctgctgctgacaagagatggcggcaagaacgacaccaatgacaccgagaccttcagacctggcggcggagacatgagggacaactggcggagcgagctgtacaagtacaaggtggtggagatcaagcctctgggcgtggcccctaccaaggccaagaggagagtggtggagagggagaagagagccgtgggcatcggcgccgtgtttctgggctttctgggagccgccggatctacaatgggagccgccagcatcacactgaccgtgcaggccagacagctgctgagcggcatcgtgcagcagcagagcaatctgctgagagccatcgaggcccagcagcacatgctgcagctgacagtgtggggcatcaagcagctgcagaccagagtgctggccatcgagcgctacctgaaggatcagcagctgctgggcatctggggctgtagcggcaagctgatctgtaccaccgccgtgccttggaatagcagctggagcaacaagagccaggaggacatctgggacaacatgacctggatgcagtgggaccgggagatcagcaactacaccgacaccatctacaggctgctggaggacagccagaaccagcaggagaagaacgagaaggacctgctggccctggacagctggaagaacctgtggaactggttcgacatcaccaactggctgtggtacatcaagatcttcatcatgattgtgggcggcctgatcggcctgagaatcatcttcgccgtgctgagcatctgatagcggccgc

SEQ ID NO: 6 - protein, 705 aa, synthetic construct
  REGION 1..705: note = Subtype C consensus Envelope protein sequence construct
MDWTWILFLVAAATRVHSRVRGILRNCQQWWIWGILGFWMLMICNVMGNLWVTVYYGVPVWKEAKTTLFCASDAKAYETEVHNVWATHACVPTDPNPQEMVLENVTENFNMWKNDMVDQMHEDIISLWDQSLKPCVKLTPLCVTLNCRNNVNNNNTMKEEIKNCSFNITTELRDKKQKVYALFYRLDIVPLNEKNNSNDYRLINCNTSAITQACPKVSFDPIPIHYCAPAGYAILKCNNKTFNGTGPCNNVSTVQCTHGIKPVVSTQLLLNGSLAEEEIIIRSENLTNNAKTIIVHLNESVEIVCTRPNNNTRKSIRIGPGQTFYATGDIIGDIRQAHCNISEEKWNKTLQRVSEKLKEHFPNKTIKFAPSSGGRLEITTHSFNCRGEFFYCNTSKLFNSTYMPNSTNNTNTTITLPCRIKQIINMWQEVGRAMYAPPIEGNITCKSNITGLLLTRDGGKNDTNDTETFRPGGGDMRDNWRSELYKYKVVEIKPLGVAPTKAKRRVVEREKRAVGIGAVFLGFLGAAGSTMGAASITLTVQARQLLSGIVQQQSNLLRAIEAQQHMLQLTVWGIKQLQTRVLAIERYLKDQQLLGIWGCSGKLICTTAVPWNSSWSNKSQEDIWDNMTWMQWDREISNYTDTIYRLLEDSQNQQEKNEKDLLALDSWKNLWNWFDITNWLWYIKIFIMIVGGLIGLRIIFAVLSI

SEQ ID NO: 7 - DNA, 2089 bp, synthetic construct
  misc_feature 1..2089: note = Subtype D consensus Envelope DNA sequence construct
  source 1..2089: mol_type = other DNA
gggcatcaagcggaattaccagcacctgtggaagtggggcaccatgctgctgggcatgctgatgacctgcagcgtggccgagaacctgtgggtgaccgtgtactacggcgtgcctgtgtggaaggaagccaccaccaccctgttctgcgccagcgatgccaagagctacaagaccgaggcccacaatatctgggccacccacgcctgcgtgcctaccgatcccaaccctcaggagatcgagctggagaacgtgaccgagaacttcaacatgtggaagaacaacatggtggagcagatgcacgaggacatcatcagcctgtgggaccagagcctgaagccttgcgtgaagctgacccctctgtgcgtgaccctgaactgcaccgacggcatgaggaacgacaccaacgataccaacgtgaccatggaggagggcgagatgaagaactgcagcttcaacatcaccaccgaagtgcgggacaagaagaagcaggtgcacgccctgttctacaagctggacgtggtgcccatcgacgacaacaacaccaacaacagcaactaccggctgatcaactgcaacaccagcgccatcacccaggcctgccccaaagtgaccttcgagcccatccccatccactactgcgcccctgccggcttcgccatcctgaagtgcaaggataagaagttcaacggcaccggcccctgcaagaatgtgagcaccgtgcagtgcacccacggcatcagacccgtggtgtccacccagctgctgctgaacggcagcctggccgaggaggagatcatcatccggagcgagaacctgaccaacaacgccaagatcatcattgtgcagctgaacgagagcgtgaccatcaattgcacccggccctacaacaatacccggaagcgcatccccatcggcctgggccaggccttctacaccaccagaggcatcatcggcgacatcagacaggcccactgcaatatcagcggagccgagtggaataagaccctgcagcaggtggccaagaagctgggcgacctgctgaacaagaccaccatcatcttcaagcctagcagcggcggcagacctagaatcaccacccacagcttcaattgtggcggcgagttcttctactgcaataccagccggctgttcaacagcacctggagcaagaacagcaccagcaactccaccaaggagaacaacaccatcaccctgccctgccggatcaagcagatcatcaatatgtggcagggagtgggcaaggccatgtacgcccctcccatcgagggcctgatcaagtgcagcagcaacatcaccggcctgctgctgaccagagatggcggagccaacaactcccacaacgagaccttcagacctggcggcggagacatgagggacaactggcggagcgagctgtacaagtacaaagtggtgaagatcgagcccctgggcgtggcccccaccagagccaagagaagagtggtggagcgggagaagagagccatcggactgggcgccatgttcctgggcttcctgggagccgccggaagcaccatgggagccgccagcctgaccctgaccgtgcaggccagacagctgctgagcggcatcgtgcagcagcagaacaacctgctgagagccattgaggcccagcagcacctgctgcagctgacagtgtggggcattaagcagctgcaggccaggattctggccgtggagcgctacctgaaggatcagcagctgctgggaatctggggctgcagcggcaagcacatctgcaccaccaccgtgccttggaatagcagctggagcaacaagagcctggacgagatctggaacaacatgacctggatggagtgggagagggagatcgacaactacaccggcctgatctacagcctgatcgaggagagccagacccagcaggagaagaacgagcaggagctgctggagctggacaagtgggccagcctgtggaactggttcagcatcacccagtggctgtggtacatcaagatcttcatcatgattgtgggcggcctgatcggcctgagaatcgtgttcgccgtgctgagcctgtgactcgag

SEQ ID NO: 8 - protein, 714 aa, synthetic construct
  REGION 1..714: note = Subtype D consensus Envelope protein sequence construct
MDWTWILFLVAAATRVHSRVRGIKRNYQHLWKWGTMLLGMLMTCSVAENLWVTVYYGVPVWKEATTTLFCASDAKSYKTEAHNIWATHACVPTDPNPQEIELENVTENFNMWKNNMVEQMHEDIISLWDQSLKPCVKLTPLCVTLNCTDGMRNDTNDTNVTMEEGEMKNCSFNITTEVRDKKKQVHALFYKLDVVPIDDNNTNNSNYRLINCNTSAITQACPKVTFEPIPIHYCAPAGFAILKCKDKKFNGTGPCKNVSTVQCTHGIRPVVSTQLLLNGSLAEEEIIIRSENLTNNAKIIIVQLNESVTINCTRPYNNTRKRIPIGLGQAFYTTRGIIGDIRQAHCNISGAEWNKTLQQVAKKLGDLLNKTTIIFKPSSGGRPRITTHSFNCGGEFFYCNTSRLFNSTWSKNSTSNSTKENNTITLPCRIKQIINMWQGVGKAMYAPPIEGLIKCSSNITGLLLTRDGGANNSHNETFRPGGGDMRDNWRSELYKYKVVKIEPLGVAPTRAKRRVVEREKRAIGLGAMFLGFLGAAGSTMGAASLTLTVQARQLLSGIVQQQNNLLRAIEAQQHLLQLTVWGIKQLQARILAVERYLKDQQLLGIWGCSGKHICTTTVPWNSSWSNKSLDEIWNNMTWMEWEREIDNYTGLIYSLIEESQTQQEKNEQELLELDKWASLWNWFSITQWLWYIKIFIMIVGGLIGLRIVFAVLSL

SEQ ID NO: 9 - DNA, 1049 bp, synthetic construct
  misc_feature 1..1049: note = Subtype B consensus Nef-Rev DNA sequence construct
  source 1..1049: mol_type = other DNA
ggatccgccaccatggactggacctggattctgttcctggtggccgctgccaccagagtgcacagcagcaagagaagcgtggtgggttggcctacagtgcgggagaggatgagaagagccgagcctgccgccgatggagtgggcgccgtgtctagagatctggagaagcacggcgccatcaccagcagcaataccgccgccaacaatgccgactgcgcctggctggaggcccaggaggaggaggaagtgggcttccctgtgagagcccaggtggccctgagagccatgacctacaaggccgccgtggatctgagccacttcctgaaggagaagggcggcctggagggcctgatctacagccagaagcggcaggacatcctggatctgtgggtgtaccacacccagggctacttccccgactggcagaattacacccctggccctggcatcagataccctctgaccttcggctggtgcttcaagctggtgcctgtggagcctgagaaagtggaggaggccaacgagggcgagaacaattctgccgcccaccctatgagcctgcacggcatggacgatcccgagagggaagtgctggtgtggaagttcgacagcaggctggccttccaccacatggccagagagctgcaccccgagtactacaaggactgccggggcaggaagagaagaagcgccggcagaagcggcgacagcgacgaggagctgctgaaaacagtgcggctgatcaagttcctgtaccagagcaaccctcctcccagccccgagggcaccagacaggcccggagaaaccggaggaggcggtggagagagaggcagcggcagatcagaagcatcagcgagtggattctgagcacctacctgggcagacccgccgagcccgtgcccctgcagctgccccccctggagagactgaccctggactgcaacgaggactgcggcaccagcggcacccagggagtgggcagcccccagatcctggtggagagccctgccgtgctggagagcggcaccaaggagtgatgagcggccgc

SEQ ID NO: 10 - protein, 341 aa, synthetic construct
  REGION 1..341: note = Subtype B consensus Nef-Rev protein sequence construct
MDWTWILFLVAAATRVHSSKRSVVGWPTVRERMRRAEPAADGVGAVSRDLEKHGAITSSNTAANNADCAWLEAQEEEEVGFPVRAQVALRAMTYKAAVDLSHFLKEKGGLEGLIYSQKRQDILDLWVYHTQGYFPDWQNYTPGPGIRYPLTFGWCFKLVPVEPEKVEEANEGENNSAAHPMSLHGMDDPEREVLVWKFDSRLAFHHMARELHPEYYKDCRGRKRRSAGRSGDSDEELLKTVRLIKFLYQSNPPPSPEGTRQARRNRRRRWRERQRQIRSISEWILSTYLGRPAEPVPLQLPPLERLTLDCNEDCGTSGTQGVGSPQILVESPAVLESGTKE

SEQ ID NO: 11 - DNA, 1863 bp, synthetic construct
  misc_feature 1..1863: note = Gag consensus DNA sequence of subtype A, B, C and D construct
  source 1..1863: mol_type = other DNA
ggatccgccaccatggactggacctggattctgtttctggtcgccgccgccacaagagtgcacagcggcgccagagccagcgtgctgtccggcggcaagctggacgcctgggagaagatcagactgaggcctggcggcaagaagaagtaccggctgaagcaccttgtgtgggccagcagagagctggagagattcgccctgaatcctggcctgctggagaccagcgagggctgtaagcagatcatcggccagctgcagcccgccctgcagaccggcagcgaggagctgagaagcctgtacaacaccgtggccaccctgtactgcgtgcacgagaagatcgaggtgaaggacaccaaggaggccctggacaagatcgaggaggagcagaacaagagcaagcagaaggcccagcaggccgccgccgacaccggcaacagcagccaggtgtcccagaactaccccatcgtgcagaatctgcagggccagatggtgcaccaggccatcagccccagaaccctgaatgcctgggtgaaggtgatcgaggagaaggccttcagccctgaggtgatccctatgttcagcgccctgagcgagggcgccacacctcaggacctgaacaccatgctgaacacagtggggggccaccaggccgccatgcagatgctgaaggataccatcaacgaggaggccgccgagtgggacagactgcaccccgtgcacgccggacctatcgcccctggccagatgagagagcccagaggcagcgacatcgccggcaccacctccaccctgcaagagcagatcggctggatgaccagcaacccccccatccctgtgggcgacatctacaagcggtggatcatcctgggcctgaacaagattgtgaggatgtacagccccgtgtccatcctggatatcaggcagggccccaaggagcccttcagagactacgtggaccggttcttcaagaccctgagagccgagcaggccagccaggacgtgaagaactggatgaccgagaccctgctggtgcagaacgccaaccccgactgtaagaccatcctgagagccctgggccctggcgccaccctggaggagatgatgaccgcctgccagggagtgggcggacccggccacaaggccagagtgctggccgaggccatgagccaggccaccaacagcaacatcatgatgcagcggggcaacttcagaggccccaggaggatcgtgaagtgcttcaactgtggcaaggagggccacatcgccagaaactgtagggcccccaggaagaagggctgctggaagtgtggcaaagaggggcaccagatgaaggactgtaccgagcggcaggccaatttcctggggaagatctggcccagccacaagggcagacccggcaatttcctgcagagcagacctgagcccaccgcccctcccgccgagagcttcggcttcggcgaggagatcacccccagccccaagcaggagcccaaggacagagagctgtaccctctggccagcctgaagagcctgttcggcaacgatcccctgagccagtacccctacgacgtgcccgattacgcctgagaattcgtaagtaagtgtcatatgggagagctcgactagactggacagccaatgacgggtaagagagtgacatttctcactaacctaagacaggagggccgtcaaagctactgcctaatccaatgacgggtaatagtgacaagaaatgtatcactccaacctaagacaggcgcagcctccgagggatgtgtcttttgttttttataattaaaaagggtgacatgtccggagccgtgctgcccggatgatgtcttggcctctgtttgctgcggccgc

SEQ ID NO: 12 - protein, 524 aa, synthetic construct
  REGION 1..524: note = Gag consensus protein sequence of subtype A, B, C and D construct
MDWTWILFLVAAATRVHSGARASVLSGGKLDAWEKIRLRPGGKKKYRLKHLVWASRELERFALNPGLLETSEGCKQIIGQLQPALQTGSEELRSLYNTVATLYCVHEKIEVKDTKEALDKIEEEQNKSKQKAQQAAADTGNSSQVSQNYPIVQNLQGQMVHQAISPRTLNAWVKVIEEKAFSPEVIPMFSALSEGATPQDLNTMLNTVGGHQAAMQMLKDTINEEAAEWDRLHPVHAGPIAPGQMREPRGSDIAGTTSTLQEQIGWMTSNPPIPVGDIYKRWIILGLNKIVRMYSPVSILDIRQGPKEPFRDYVDRFFKTLRAEQASQDVKNWMTETLLVQNANPDCKTILRALGPGATLEEMMTACQGVGGPGHKARVLAEAMSQATNSNIMMQRGNFRGPRRIVKCFNCGKEGHIARNCRAPRKKGCWKCGKEGHQMKDCTERQANFLGKIWPSHKGRPGNFLQSRPEPTAPPAESFGFGEEITPSPKQEPKDRELYPLASLKSLFGNDPLSQYPYDVPDYA

SEQ ID NO: 13 - DNA, 43 bp, synthetic construct
  misc_feature 1..43: note = IgE Primer Sequence 1
  source 1..43: mol_type = other DNA
gtcgctccgctagcttgtgggtcacagtctattatggggtacc

SEQ ID NO: 14 - DNA, 35 bp, synthetic construct
  misc_feature 1..35: note = IgE Primer Sequence 2
  source 1..35: mol_type = other DNA
ggtcggatccttactccaccactctcctttttgcc

SEQ ID NO: 15 - protein, 17 aa, synthetic construct
  REGION 1..17: note = IgE leader sequence
MDWTWILFLVAAATRVH

SEQ ID NO: 16 - protein, 692 aa, synthetic construct
  REGION 1..692: note = Subtype A consensus Envelope protein sequence
SRVMGIQRNCQHLWRWGTMILGMIIICSAAENLWVTVYYGVPVWKDAETTLFCASDAKAYDTEVHNVWATHACVPTDPNPQEINLENVTEEFNMWKNNMVEQMHTDIISLWDQSLKPCVKLTPLCVTLNCSNVNVTTNIMKGEIKNCSFNMTTELRDKKQKVYSLFYKLDVVQINKSNSSSQYRLINCNTSAITQACPKVSFEPIPIHYCAPAGFAILKCKDKEFNGTGPCKNVSTVQCTHGIKPVVSTQLLLNGSLAEEEVMIRSENITNNAKNIIVQLTKPVKINCTRPNNNTRKSIRIGPGQAFYATGDIIGDIRQAHCNVSRTEWNETLQKVAKQLRKYFNNKTIIFTNSSGGRLRITTHSFNCGGEFFYCNTSGLFNSTWNGNGTKKKNSTESNDTITLPCRIKQIINMWQRVGQAMYAPPIQGVIRCESNITGLLLTRDGGDNNSKNETFRPGGGDMRDNWRSELYKYKVVKIEPLGVAPTKAKRRVVEREKRAVGIGAVFLGFLGAAGSTMGAASITLTVQARQLLSGIVQQQSNLLRAIEAQQHLLKLTVWGIKQLQARVLAVERYLKDQQLLGIWGCSGKLICTTNVPWNSSWSNKSQSEIWDNMTWLQWDKEISNYTDIIYNLIEESQNQQEKNEQDLLALDKWANLWNWFDISNWLWYIKIFIMIVGGLIGLRIVFAVLSV

SEQ ID NO: 17 - protein, 697 aa, synthetic construct
  REGION 1..697: note = Subtype B consensus Envelope protein sequence
RVKGIRKNYQHLWRWGTMLLGMLMICSAAEKLWVTVYYGVPVWKEATTTLFCASDAKAYDTEVHNVWATHACVPTDPNPQEVVLENVTENFNMWKNNMVEQMHEDIISLWDQSLKPCVKLTPLCVTLNCTDLSGEKMEKGEIKNCSFNITTSIRDKVQKEYALFYKLDVVPIDNDNTSYRLISCNTSVITQACPKVSFEPIPIHYCAPAGFAILKCNDKKFNGTGPCTNVSTVQCTHGIRPVVSTQLLLNGSLAEEEVVIRSENFTNNAKTIIVQLNESVEINCTRPNNNTRKSIHIGPGQAFYTTGEIIGDIRQAHCNISRAKWNNTLKQIVKKLREQFGNKTIVFNQSSGGRPRIVMHSFNCGGEFFYCNTTQLFNSTWNVNGTWNNNTEGNDTITLPCRIKQIINMWQEVGKAMYAPPIRGQIRCSSNITGLLLTRDGGNNNTNETEIFRPGGGDMRDNWRSELYKYKVVKIEPLGVAPTKAKRRVVQREKRAVGIGAMFLGFLGAAGSTMGAASMTLTVQARQLLSGIVQQQNNLLRAIEAQQHLLQLTVWGIKQLQARVLAVERYLKDQQLLGIWGCSGKLICTTTVPWNASWSNKSLDEIWDNMTWMEWEREIDNYTSLIYTLIEESQNQQEKNEQELLELDKWASLWNWFDITNWLWYIKIFIMIVGGLIGLRIVFAVLSIYPYDVPDYA

SEQ ID NO: 18 - protein, 687 aa, synthetic construct
  REGION 1..687: note = Subtype C consensus Envelope protein sequence
RVRGILRNCQQWWIWGILGFWMLMICNVMGNLWVTVYYGVPVWKEAKTTLFCASDAKAYETEVHNVWATHACVPTDPNPQEMVLENVTENFNMWKNDMVDQMHEDIISLWDQSLKPCVKLTPLCVTLNCRNNVNNNNTMKEEIKNCSFNITTELRDKKQKVYALFYRLDIVPLNEKNNSNDYRLINCNTSAITQACPKVSFDPIPIHYCAPAGYAILKCNNKTFNGTGPCNNVSTVQCTHGIKPVVSTQLLLNGSLAEEEIIIRSENLTNNAKTIIVHLNESVEIVCTRPNNNTRKSIRIGPGQTFYATGDIIGDIRQAHCNISEEKWNKTLQRVSEKLKEHFPNKTIKFAPSSGGRLEITTHSFNCRGEFFYCNTSKLFNSTYMPNSTNNTNTTITLPCRIKQIINMWQEVGRAMYAPPIEGNITCKSNITGLLLTRDGGKNDTNDTETFRPGGGDMRDNWRSELYKYKVVEIKPLGVAPTKAKRRVVEREKRAVGIGAVFLGFLGAAGSTMGAASITLTVQARQLLSGIVQQQSNLLRAIEAQQHMLQLTVWGIKQLQTRVLAIERYLKDQQLLGIWGCSGKLICTTAVPWNSSWSNKSQEDIWDNMTWMQWDREISNYTDTIYRLLEDSQNQQEKNEKDLLALDSWKNLWNWFDITNWLWYIKIFIMIVGGLIGLRIIFAVLSI

SEQ ID NO: 19 - protein, 696 aa, synthetic construct
  REGION 1..696: note = Subtype D consensus Envelope protein sequence
RVRGIKRNYQHLWKWGTMLLGMLMTCSVAENLWVTVYYGVPVWKEATTTLFCASDAKSYKTEAHNIWATHACVPTDPNPQEIELENVTENFNMWKNNMVEQMHEDIISLWDQSLKPCVKLTPLCVTLNCTDGMRNDTNDTNVTMEEGEMKNCSFNITTEVRDKKKQVHALFYKLDVVPIDDNNTNNSNYRLINCNTSAITQACPKVTFEPIPIHYCAPAGFAILKCKDKKFNGTGPCKNVSTVQCTHGIRPVVSTQLLLNGSLAEEEIIIRSENLTNNAKIIIVQLNESVTINCTRPYNNTRKRIPIGLGQAFYTTRGIIGDIRQAHCNISGAEWNKTLQQVAKKLGDLLNKTTIIFKPSSGGRPRITTHSFNCGGEFFYCNTSRLFNSTWSKNSTSNSTKENNTITLPCRIKQIINMWQGVGKAMYAPPIEGLIKCSSNITGLLLTRDGGANNSHNETFRPGGGDMRDNWRSELYKYKVVKIEPLGVAPTRAKRRVVEREKRAIGLGAMFLGFLGAAGSTMGAASLTLTVQARQLLSGIVQQQNNLLRAIEAQQHLLQLTVWGIKQLQARILAVERYLKDQQLLGIWGCSGKHICTTTVPWNSSWSNKSLDEIWNNMTWMEWEREIDNYTGLIYSLIEESQTQQEKNEQELLELDKWASLWNWFSITQWLWYIKIFIMIVGGLIGLRIVFAVLSL

SEQ ID NO: 20 - protein, 323 aa, synthetic construct
  REGION 1..323: note = Subtype B consensus Nef-Rev protein sequence
SKRSVVGWPTVRERMRRAEPAADGVGAVSRDLEKHGAITSSNTAANNADCAWLEAQEEEEVGFPVRAQVALRAMTYKAAVDLSHFLKEKGGLEGLIYSQKRQDILDLWVYHTQGYFPDWQNYTPGPGIRYPLTFGWCFKLVPVEPEKVEEANEGENNSAAHPMSLHGMDDPEREVLVWKFDSRLAFHHMARELHPEYYKDCRGRKRRSAGRSGDSDEELLKTVRLIKFLYQSNPPPSPEGTRQARRNRRRRWRERQRQIRSISEWILSTYLGRPAEPVPLQLPPLERLTLDCNEDCGTSGTQGVGSPQILVESPAVLESGTKE

SEQ ID NO: 21 - protein, 506 aa, synthetic construct
  REGION 1..506: note = Gag consensus protein sequence of subtype A, B, C and D
GARASVLSGGKLDAWEKIRLRPGGKKKYRLKHLVWASRELERFALNPGLLETSEGCKQIIGQLQPALQTGSEELRSLYNTVATLYCVHEKIEVKDTKEALDKIEEEQNKSKQKAQQAAADTGNSSQVSQNYPIVQNLQGQMVHQAISPRTLNAWVKVIEEKAFSPEVIPMFSALSEGATPQDLNTMLNTVGGHQAAMQMLKDTINEEAAEWDRLHPVHAGPIAPGQMREPRGSDIAGTTSTLQEQIGWMTSNPPIPVGDIYKRWIILGLNKIVRMYSPVSILDIRQGPKEPFRDYVDRFFKTLRAEQASQDVKNWMTETLLVQNANPDCKTILRALGPGATLEEMMTACQGVGGPGHKARVLAEAMSQATNSNIMMQRGNFRGPRRIVKCFNCGKEGHIARNCRAPRKKGCWKCGKEGHQMKDCTERQANFLGKIWPSHKGRPGNFLQSRPEPTAPPAESFGFGEEITPSPKQEPKDRELYPLASLKSLFGNDPLSQYPYDVPDYA

SEQ ID NO: 22 - DNA, 818 bp, synthetic construct
  misc_feature 1..818: note = HPV genotype 16 E6-E7 DNA sequence
  source 1..818: mol_type = other DNA
gaattcgccaccatggactggacctggatcctgttcctggtggccgccgccacacgggtgcacagcttccaggacccccaggagagcggcagaaagctgcctcagctgtgtaccgagctgcagaccaccatccacgacatcatcctggagtgtgtgtactgtaagcagcagctgctgaggagagaggtgtacgaccgggacctgtgtatcgtgtacagggacggcaatccctacgccgtgtgtgacaagtgcctgaagttctacagcaagatcagcgagtaccggcactactgctacagcctgtacggcaccaccctggagcagcagtacaacaagcccctgtgtgacctgctgatccggtgtatcaactgccagaagcccctgcagagacacctggacaagaagcagcggttccacaacatcaggggcagatggaccggcagatgtatgagctgctgccggagcagcagaaccagaagggagacccagctgagaggccggaagagaagaagccacggcgatacccccaccctgcacgagtacatgctggacctgcagcctgagaccaccgatctgtacggctacggccagctgaatgacagcagcgaggaggaggatgagatcgacggccctgccggccaggccgagcccgacagagcccactacaacatcgtgaccttttgctgtaagtgtgacagcaccctgagactgtgcgtgcagagcacccacgtggacatcagaaccctggaggatctgctgatgggcaccctgggcatcgtgtgtcccatctgctcccagaaaccctgatgagcggccgc

SEQ ID NO: 23 - protein, 264 aa, synthetic construct
  REGION 1..264: note = HPV genotype 16 E6-E7 protein sequence
MDWTWILFLVAAATRVHSFQDPQESGRKLPQLCTELQTTIHDIILECVYCKQQLLRREVYDRDLCIVYRDGNPYAVCDKCLKFYSKISEYRHYCYSLYGTTLEQQYNKPLCDLLIRCINCQKPLQRHLDKKQRFHNIRGRWTGRCMSCCRSSRTRRETQLRGRKRRSHGDTPTLHEYMLDLQPETTDLYGYGQLNDSSEEEDEIDGPAGQAEPDRAHYNIVTFCCKCDSTLRLCVQSTHVDIRTLEDLLMGTLGIVCPICSQKP

SEQ ID NO: 24 - protein, 15 aa, synthetic construct
  REGION 1..15: note = HPV E6 immunodominant epitope
LCIVYRDGNPYAVCD

SEQ ID NO: 25 - protein, 15 aa, synthetic construct
  REGION 1..15: note = HPV E7 immunodominant epitope
AEPDRAHYNIVTFCC

SEQ ID NO: 26 - protein, 142 aa, synthetic construct
  REGION 1..142: note = HPV E6 consensus sequence
FQDPQESGRKLPQLCTELQTTIHDIILECVYCKQQLLRREVYDRDLCIVYRDGNPYAVCDKCLKFYSKISEYRHYCYSLYGTTLEQQYNKPLCDLLIRCINCQKPLQRHLDKKQRFHNIRGRWTGRCMSCCRSSRTRRETQL

SEQ ID NO: 27 - protein, 97 aa, synthetic construct
  REGION 1..97: note = HPV E7 consensus sequence
HGDTPTLHEYMLDLQPETTDLYGYGQLNDSSEEEDEIDGPAGQAEPDRAHYNIVTFCCKCDSTLRLCVQSTHVDIRTLEDLLMGTLGIVCPICSQKP

SEQ ID NO: 28 - protein, 18 aa, synthetic construct
  REGION 1..18: note = IgE Leader Sequence
MDWTWILFLVAAATRVHS

SEQ ID NO: 29 - protein, 7 aa, synthetic construct
  REGION 1..7: note = Proteolytic Cleavage Sequence
RGRKRRS

SEQ ID NO: 30 - DNA, 1766 bp, synthetic construct
  misc_feature 1..1766: note = HCV genotype 1a and 1b consensus E1-E2 DNA sequence
  source 1..1766: mol_type = other DNA
gaattcgccaccatggactggacctggatcctgttcctggtggccgctgcaacacgggtgcacagctaccaagtgaggaatagcagcggcctgtaccacgtgaccaacgactgctccaacagcagcatcgtgtacgaggccgccgacatgatcatgcacacccccggctgtgtgccctgtgtgagagagggcaacagctccagatgctgggtggccctgacccctaccgtggccgccagagatggcagcctgcccaccaccaccctgaggagacacgtggacctgcttgtgggcagcgccaccctgtgtagcgccatgtatgtgggcgatctgtgtggcagcgtgtttcttgtgggccagctgttcaccttcagccccagaaggcactggaccgtgcaggactgtaactgctccatctaccccggccacatcaccggccacagaatggcctgggacatgatgatgaactggagccctaccaccgccctggtggtgtcccagctgctgagaatccctcaggccatcgtggacatggtggccggagcccactggggcgtgctggccggcatcgcctacttcagcatggtgggcaactgggccaaggtgctcgtggtgctgctgctgttcgccggcgtggacggcagaggcaggaagagaaggagcgagacccacgtgaccggcggcaccgccggcagaaccacagccggccttgtgggcctgttcacccctggcgccaagcagaacatccagctgatcaacaccaacggcagctggcacatcaacagcaccgccctgaactgtaacgacagcctgaacaccggctggctggccggcctgttctaccagcacaagttcaacagcagcggctgccccgagagaatggccagctgtagacccctggatgagttcgcccagggctggggccccatcacctacgccaatggcagcggccctgaccagagaccctactgctggcactacgcccccagaccctgtggcatcgtgcccgccaagagcgtgtgtggccccgtgtactgcttcacccctagccccgtggttgtgggcaccaccgacagaagcggagcccccacctacagctggggcgagaacgagaccgacgtgctggtgctgaacaacaccagaccccccctgggcaattggttcggctgtacctggatgaacagcaccggcttcaccaaagtgtgtggcgcccctccctgtgtgatcggcggagtgggcaacaacaccctgacctgccccaccgactgcttcagaaagcaccccgaggccacctactccagatgtggcagcggaccttggctgacccccagatgtatggtggactacccctacaggctgtggcactacccctgtaccgtgaacttcaccatcttcaaagtgaggatgtatgtggggggcgtggagcacagactggaggccgcctgtaattggaccaggggcgagagatgtgacctggaggaccgggatagaagcgagctgtcccctctgctgctgtccaccaccgagtggcaggtgctgccttgtagcttcaccaccctgcccgccctgagcaccggcctgatccacctgcaccagaacatcgtggacgtgcagtacctgtacggagtgggctctagcatcgtgtcctgggccatcaagtgggagtacgtggtgctgctgttcctgctgctggccgacgccagagtgtgtagctgcctgtggatgatgctgctgatcagccaggccgaggcctgatgagcggccgc

SEQ ID NO: 31 - protein, 580 aa, synthetic construct
  REGION 1..580: note = HCV genotype 1a and 1b consensus E1-E2 protein sequence
MDWTWILFLVAAATRVHSYQVRNSSGLYHVTNDCSNSSIVYEAADMIMHTPGCVPCVREGNSSRCWVALTPTVAARDGSLPTTTLRRHVDLLVGSATLCSAMYVGDLCGSVFLVGQLFTFSPRRHWTVQDCNCSIYPGHITGHRMAWDMMMNWSPTTALVVSQLLRIPQAIVDMVAGAHWGVLAGIAYFSMVGNWAKVLVVLLLFAGVDGRGRKRRSETHVTGGTAGRTTAGLVGLFTPGAKQNIQLINTNGSWHINSTALNCNDSLNTGWLAGLFYQHKFNSSGCPERMASCRPLDEFAQGWGPITYANGSGPDQRPYCWHYAPRPCGIVPAKSVCGPVYCFTPSPVVVGTTDRSGAPTYSWGENETDVLVLNNTRPPLGNWFGCTWMNSTGFTKVCGAPPCVIGGVGNNTLTCPTDCFRKHPEATYSRCGSGPWLTPRCMVDYPYRLWHYPCTVNFTIFKVRMYVGGVEHRLEAACNWTRGERCDLEDRDRSELSPLLLSTTEWQVLPCSFTTLPALSTGLIHLHQNIVDVQYLYGVGSSIVSWAIKWEYVVLLFLLLADARVCSCLWMMLLISQAEA

SEQ ID NO: 32 - protein, 192 aa, synthetic construct
  REGION 1..192: note = HCV E1 consensus sequence
YQVRNSSGLYHVTNDCSNSSIVYEAADMIMHTPGCVPCVREGNSSRCWVALTPTVAARDGSLPTTTLRRHVDLLVGSATLCSAMYVGDLCGSVFLVGQLFTFSPRRHWTVQDCNCSIYPGHITGHRMAWDMMMNWSPTTALVVSQLLRIPQAIVDMVAGAHWGVLAGIAYFSMVGNWAKVLVVLLLFAGVDG

SEQ ID NO: 33 - protein, 363 aa, synthetic construct
  REGION 1..363: note = HCV E2 consensus sequence
ETHVTGGTAGRTTAGLVGLFTPGAKQNIQLINTNGSWHINSTALNCNDSLNTGWLAGLFYQHKFNSSGCPERMASCRPLDEFAQGWGPITYANGSGPDQRPYCWHYAPRPCGIVPAKSVCGPVYCFTPSPVVVGTTDRSGAPTYSWGENETDVLVLNNTRPPLGNWFGCTWMNSTGFTKVCGAPPCVIGGVGNNTLTCPTDCFRKHPEATYSRCGSGPWLTPRCMVDYPYRLWHYPCTVNFTIFKVRMYVGGVEHRLEAACNWTRGERCDLEDRDRSELSPLLLSTTEWQVLPCSFTTLPALSTGLIHLHQNIVDVQYLYGVGSSIVSWAIKWEYVVLLFLLLADARVCSCLWMMLLISQAEA

SEQ ID NO: 34 - DNA, 3512 bp, Homo sapiens
  source 1..3512: mol_type = unassigned DNA
ggtaccgaattcgccaccatggactggacctggatcctgttcctggtggccgctgccacaagagtgcacagccccagggcccccaggtgcagagccgtgcggagcctgctgcggagccactaccgggaggtgctgcccctggccaccttcgtgcggaggctgggccctcaggggtggcggctggtgcagagaggcgaccctgccgccttcagagccctggtggcccagtgcctggtgtgcgtgccctgggacgccagacctccccctgccgcccctagcttccggcaggtgtcctgcctgaaagaactggtggcccgggtgctgcagcggctgtgcgagaggggcgccaagaacgtgctggccttcggcttcgccctgctggacggcgccagaggcggccctcccgaggccttcaccacctccgtgagaagctacctgcccaacaccgtgaccgacgccctgagaggcagcggcgcttggggcctgctgctgcgcagagtgggcgacgacgtgctggtgcacctgctggccagatgcgccctgttcgtgctggtcgcccccagctgcgcctaccaggtgtgcggcccacccctgtaccagctgggagccgccacccaggccagaccccctcctcacgcctccggccccaggcggagactgggctgcgagcgggcctggaaccacagcgtgcgggaggccggcgtgcccctgggcctgccagcccctggcgccagaagaaggggcggcagcgccagcagaagcctgcccctgcccaagcggcccagacgcggagccgcccctgagcccgagagaacccccgtgggccagggctcttgggcccaccctggccggaccagaggccccagcgaccggggcttctgcgtggtgtcccccgccagacccgccgaggaagccacctccctggaaggcgccctgagcggcaccaggcacagccaccccagcgtgggccgccagcaccacgccggaccccccagcacctccaggccccccaggccctgggacaccccttgcccccctgtgtacgccgagaccaagcacttcctgtacagcagcggcgacaaagagcagctgcggcccagcttcctgctgtccagcctgaggccctccctgaccggcgctaggcgcctggtggagaccatctttctgggcagccggccctggatgcccggcacccccaggcggctgcccaggctgccccagcggtactggcagatgaggcctctgttcctggaactgctgggcaaccacgcccagtgcccctacggcgtgctgctgaaaacccactgccccctgagagccgccgtgaccccagccgccggagtgtgcgccagagagaagcctcagggcagcgtggccgctcccgaggaagaggacaccgaccccagacgcctggtgcagctgctgcggcagcacagcagcccttggcaggtgtacggcttcgtgcgggcctgcctgagaaggctggtgccccctggcctgtggggcagcaggcacaacgagcggcggtttctgcggaacaccaagaagttcatcagcctggggaagcacgccaagctgtccctgcaggaactgacctggaagatgagcgtgcggggctgcgcctggctgagaagatcccctggcgtgggctgcgtgcctgccgccgagcaccggctgcgggaggaaatcctggccaagttcctgcactggctgatgagcgtgtacgtggtggagctgctgagatccttcttctacgtgaccgagaccaccttccagaagaactacctgttcttctaccggaagagcgtgtggagcaagctgcagagcatcggcatccggcagcacctgaagcgggtgcagctgagagagctgtccgaggccgaagtgaggcagcaccgggaggccagacctgccctgctgaccagccggctgcggttcatccccaagcccgacggcctgcggcccatcgtgaacatggactacgtggtgggcgccaggaccttccggcgggagaagcgggccgagcggctgacctcgagggtgaaggccctgttcagcgtgctgaactacgagcgggccaggcggccaggcctgctgggcgccagcgtgctgggcctggacgacatccaccgggcctggcggaccttcgtgctgagagtgcgggcccaggacccccctcccgagctgtacttcgtgaaggtggacgtgacaggcgcctacgacaccatcccccaggaccggctgaccgaggtgatcgccagcatcatcaagccccagaacacctactgcgtgcggagatacgccgtggtgcagaaggccgcccacggccacgtgcggaaggccttcaagagccacgtgagcaccctgaccgacctgcagccctacatgcggcagttcgtggcccacctgcaggaaaccagccccctgcgggatgccgtggtgatcgagcagagcagcagcctgaacgaggccagcagcggcctgttcgacgtgttcctgagattcatgtgccaccacgccgtgcggatccggggcaagagctacgtgcagtgccagggcatcccacagggcagcatcctgtccaccctgctgtgctccctgtgctacggcgacatggaaaacaagctgttcgccggcatcaggcgggacggactgctgctgagactggtggacgacttcctgctggtgaccccccacctgacccacgccaagacctttctgcggaccctggtgcgcggcgtgcccgagtacggctgcgtggtgaacctgagaaagaccgtggtgaacttccccgtggaggacgaggccctgggcggcacagccttcgtgcagatgcctgcccatggactgttcccttggtgcgggctgctgctggacacccggaccctggaagtgcagagcgactacagcagctacgcccggaccagcatccgggcctccctgaccttcaacaggggcttcaaggccggcaggaacatgcggcggaagctgtttggcgtgctgcggctgaagtgccacagcctgtttctgtacctgcaggtgaacagcctgcagaccgtgtgcaccaacatctacaagatcctgctgctgcaggcctaccggttccacgcctgcgtgctgcagctgccctttcaccagcaggtgtggaagaaccctaccttcttcctgcgggtgatcagcgacaccgccagcctgtgctacagcatcctgaaggccaagaacgccggcatgagcctgggcgccaagggagccgccggacctctgcccagcgaggccgtgcagtggctgtgccaccaggcctttctgctgaagctgacccggcaccgggtgacctacgtgcccctgctgggcagcctgcggaccgcccagacccagctgtcccggaagctgcctggcaccaccctgacagccctggaagccgccgccaaccccgccctgccctccgacttcaagaccatcctggactacccctacgacgtgcccgactacgcctgatgagcggccgcgagctc

SEQ ID NO: 35 - protein, 1158 aa, Homo sapiens
MDWTWILFLVAAATRVHSPRAPRCRAVRSLLRSHYREVLPLATFVRRLGPQGWRLVQRGDPAAFRALVAQCLVCVPWDARPPPAAPSFRQVSCLKELVARVLQRLCERGAKNVLAFGFALLDGARGGPPEAFTTSVRSYLPNTVTDALRGSGAWGLLLRRVGDDVLVHLLARCALFVLVAPSCAYQVCGPPLYQLGAATQARPPPHASGPRRRLGCERAWNHSVREAGVPLGLPAPGARRRGGSASRSLPLPKRPRRGAAPEPERTPVGQGSWAHPGRTRGPSDRGFCVVSPARPAEEATSLEGALSGTRHSHPSVGRQHHAGPPSTSRPPRPWDTPCPPVYAETKHFLYSSGDKEQLRPSFLLSSLRPSLTGARRLVETIFLGSRPWMPGTPRRLPRLPQRYWQMRPLFLELLGNHAQCPYGVLLKTHCPLRAAVTPAAGVCAREKPQGSVAAPEEEDTDPRRLVQLLRQHSSPWQVYGFVRACLRRLVPPGLWGSRHNERRFLRNTKKFISLGKHAKLSLQELTWKMSVRGCAWLRRSPGVGCVPAAEHRLREEILAKFLHWLMSVYVVELLRSFFYVTETTFQKNYLFFYRKSVWSKLQSIGIRQHLKRVQLRELSEAEVRQHREARPALLTSRLRFIPKPDGLRPIVNMDYVVGARTFRREKRAERLTSRVKALFSVLNYERARRPGLLGASVLGLDDIHRAWRTFVLRVRAQDPPPELYFVKVDVTGAYDTIPQDRLTEVIASIIKPQNTYCVRRYAVVQKAAHGHVRKAFKSHVSTLTDLQPYMRQFVAHLQETSPLRDAVVIEQSSSLNEASSGLFDVFLRFMCHHAVRIRGKSYVQCQGIPQGSILSTLLCSLCYGDMENKLFAGIRRDGLLLRLVDDFLLVTPHLTHAKTFLRTLVRGVPEYGCVVNLRKTVVNFPVEDEALGGTAFVQMPAHGLFPWCGLLLDTRTLEVQSDYSSYARTSIRASLTFNRGFKAGRNMRRKLFGVLRLKCHSLFLYLQVNSLQTVCTNIYKILLLQAYRFHACVLQLPFHQQVWKNPTFFLRVISDTASLCYSILKAKNAGMSLGAKGAAGPLPSEAVQWLCHQAFLLKLTRHRVTYVPLLGSLRTAQTQLSRKLPGTTLTALEAAANPALPSDFKTILDYPYDVPDYA

SEQ ID NO: 36 - DNA, 1707 bp, synthetic construct
  misc_feature 1..1707: note = Influenza H5N1 HA consensus sequence
  source 1..1707: mol_type = other DNA
atggaaaagatcgtgctgctgttcgccatcgtgagcctggtgaagagcgaccagatctgcatcggctaccacgccaacaacagcaccgagcaggtggacaccatcatggaaaaaaacgtgaccgtgacccacgcccaggacatcctggaaaagacccacaacggcaagctgtgcgacctggacggcgtgaagcccctgatcctgcgggactgcagcgtggccggctggctgctgggcaaccccatgtgcgacgagttcatcaacgtgcccgagtggagctacatcgtggagaaggccaaccccgtgaacgacctgtgctaccccggcgacttcaacgactacgaggaactgaagcacctgctgtcccggatcaaccacttcgagaagatccagatcatccccaagagcagctggtccagccacgaggccagcctgggcgtgagcagcgcctgcccataccagggcaagtccagcttcttccggaacgtggtgtggctgatcaagaagaacagcacctaccccaccatcaagcggagctacaacaacaccaaccaggaagatctgctggtcctgtggggcatccaccaccccaacgacgccgccgagcagaccaagctgtaccagaaccccaccacctacatcagcgtgggcaccagcaccctgaaccagcggctggtgccccggatcgccacccggtccaaggtgaacggccagagcggccggatggaattcttctggaccatcctgaagcccaacgatgccatcaacttcgagagcaacggcaacttcatcgcccccgagtacgcctacaagatcgtgaagaagggcgacagcaccatcatgaagagcgagctggaatacggcaactgcaacaccaagtgccagacccccatgggcgccatcaacagcagcatgcccttccacaacatccaccccctgaccatcggcgagtgccccaagtacgtgaagagcaacaggctggtgctggccaccggcctgcggaacagcccccagcgggagcggcgggccgccgcccggggcctgttcggcgccatcgccggcttcatcgagggcggctggcagggcatggtggacgggtggtacggctaccaccacagcaatgagcagggcagcggctacgccgccgacaaagagagcacccagaaggccatcgacggcgtcaccaacaaggtgaacagcatcatcgacaagatgaacacccagttcgaggccgtgggccgggagttcaacaacctggaacggcggatcgagaacctgaacaagaaaatggaagatggcttcctggacgtgtggacctacaacgccgagctgctggtgctgatggaaaacgagcggaccctggacttccacgacagcaacgtgaagaacctgtacgacaaagtgcggctgcagctgcgggacaacgccaaagagctgggcaacggctgcttcgagttctaccacaagtgcgacaacgagtgcatggaaagcgtgcggaacggcacctacgactacccccagtacagcgaggaagcccggctgaagcgggaggaaatcagcggcgtgaaactggaaagcatcggcatctaccagatcctgagcatctacagcaccgtggccagcagcctggccctggccatcatggtggccggcctgagcctgtggatgtgcagcaacggcagcctgcagtgccggatctgcatctag

SEQ ID NO: 37 - protein, 568 aa, synthetic construct
  REGION 1..568: note = Influenza H5N1 HA consensus sequence
MEKIVLLFAIVSLVKSDQICIGYHANNSTEQVDTIMEKNVTVTHAQDILEKTHNGKLCDLDGVKPLILRDCSVAGWLLGNPMCDEFINVPEWSYIVEKANPVNDLCYPGDFNDYEELKHLLSRINHFEKIQIIPKSSWSSHEASLGVSSACPYQGKSSFFRNVVWLIKKNSTYPTIKRSYNNTNQEDLLVLWGIHHPNDAAEQTKLYQNPTTYISVGTSTLNQRLVPRIATRSKVNGQSGRMEFFWTILKPNDAINFESNGNFIAPEYAYKIVKKGDSTIMKSELEYGNCNTKCQTPMGAINSSMPFHNIHPLTIGECPKYVKSNRLVLATGLRNSPQRERRAAARGLFGAIAGFIEGGWQGMVDGWYGYHHSNEQGSGYAADKESTQKAIDGVTNKVNSIIDKMNTQFEAVGREFNNLERRIENLNKKMEDGFLDVWTYNAELLVLMENERTLDFHDSNVKNLYDKVRLQLRDNAKELGNGCFEFYHKCDNECMESVRNGTYDYPQYSEEARLKREEISGVKLESIGIYQILSIYSTVASSLALAIMVAGLSLWMCSNGSLQCRICI

SEQ ID NO: 38 - DNA, 1466 bp, synthetic construct
  misc_feature 1..1466: note = Influenza H1N1&H5N1 NA consensus Sequence
  source 1..1466: mol_type = other DNA
ggtaccgaattcgccaccatggactggacctggatcctgttcctggtggccgctgccacccgggtgcacagcatgaaccccaaccagaagatcatcaccatcggcagcatctgcatggtgatcggcatcgtgagcctgatgctgcagatcggcaacatgatcagcatctgggtgtcccacagcatccagaccggcaaccagcaccaggccgagcccatcagcaacaccaactttctgaccgagaaggccgtggccagcgtgaccctggccggcaacagcagcctgtgccccatcagcggctgggccgtgtacagcaaggacaacagcatccggatcggcagcaagggcgacgtgttcgtgatccgggagcccttcatcagctgcagccacctggaatgccggaccttcttcctgacccagggggccctgctgaacgacaagcacagcaacggcaccgtgaaggacagaagcccctaccggaccctgatgagctgccccgtgggcgaggcccccagcccctacaacagccggttcgagagcgtggcctggtccgccagcgcctgccacgacggcaccagctggctgaccatcggcatcagcggccctgacaacggcgccgtggccgtgctgaagtacaacggcatcatcaccgacaccatcaagagctggcggaacaacatcctgcggacccaggaaagcgagtgcgcctgcgtgaacggcagctgcttcaccgtgatgaccgacggccccagcaacggccaggccagctacaagatcttcaagatggaaaagggcaaggtggtgaagagcgtggagctggacgcccccaactaccactacgaggaatgcagctgctaccccgacgccggcgagatcacctgcgtgtgccgggacaactggcacggcagcaaccggccctgggtgtccttcaaccagaacctggaataccagatcggctacatctgcagcggcgtgttcggcgacaaccccaggcccaacgatggcaccggcagctgcggccctgtgagcgccaacggcgcctacggcgtgaagggcttcagcttcaagtacggcaacggcgtgtggatcggccggaccaagagcaccaacagcagatccggcttcgagatgatctgggaccccaacggctggaccgagaccgacagcagcttcagcgtgaagcaggacatcgtggccatcaccgactggtccggctacagcggcagcttcgtgcagcaccccgagctgaccggcctggactgcatccggccctgcttttgggtggagctgatcagaggcaggcccaaagagagcaccatctggaccagcggcagcagcatcagcttttgcggcgtgaacagcgacaccgtgagctggtcctggcccgacggcgccgagctgcccttcaccatcgacaagtacccctacgacgtgcccgactacgcctgatgagcggccgcgagctc

SEQ ID NO: 39 - protein, 476 aa, synthetic construct
  REGION 1..476: note = Influenza H1N1&H5N1 NA consensus sequence
MDWTWILFLVAAATRVHSMNPNQKIITIGSICMVIGIVSLMLQIGNMISIWVSHSIQTGNQHQAEPISNTNFLTEKAVASVTLAGNSSLCPISGWAVYSKDNSIRIGSKGDVFVIREPFISCSHLECRTFFLTQGALLNDKHSNGTVKDRSPYRTLMSCPVGEAPSPYNSRFESVAWSASACHDGTSWLTIGISGPDNGAVAVLKYNGIITDTIKSWRNNILRTQESECACVNGSCFTVMTDGPSNGQASYKIFKMEKGKVVKSVELDAPNYHYEECSCYPDAGEITCVCRDNWHGSNRPWVSFNQNLEYQIGYICSGVFGDNPRPNDGTGSCGPVSANGAYGVKGFSFKYGNGVWIGRTKSTNSRSGFEMIWDPNGWTETDSSFSVKQDIVAITDWSGYSGSFVQHPELTGLDCIRPCFWVELIRGRPKESTIWTSGSSISFCGVNSDTVSWSWPDGAELPFTIDKYPYDVPDYA

SEQ ID NO: 40 - DNA, 875 bp, synthetic construct
  misc_feature 1..875: note = Influenza H1N1&H5N1 M1 consensus sequence
  source 1..875: mol_type = other DNA
ggtaccggatccgccaccatggactggacctggattctgttcctggtggccgctgccacccgggtgcacagcatgagcctgctgaccgaggtggagacctacgtgctgtccatcatccccagcggccctctgaaggccgagatcgcccagcggctggaagatgtgttcgccggcaagaacaccgacctggaagccctgatggaatggctgaaaacccggcccatcctgagccccctgaccaagggcatcctgggcttcgtgttcaccctgaccgtgcccagcgagcggggcctgcagcggcggagattcgtgcagaacgccctgaacggcaacggcgaccccaacaacatggaccgggccgtgaagctgtacaagaagctgaagcgggagatcaccttccacggcgccaaagaggtggccctgagctacagcacaggcgccctggccagctgcatgggcctgatctacaaccggatgggcaccgtgaccaccgaggtggccttcggcctggtgtgcgccacctgcgagcagatcgccgacagccagcacagatcccaccggcagatggccaccaccaccaaccccctgatccggcacgagaaccggatggtcctggcctccaccaccgccaaggccatggaacagatggccggcagcagcgagcaggccgccgaagccatggaagtggccagccaggccaggcagatggtgcaggccatgcggaccatcggcacccaccccagcagcagcgccggactgcgggacgacctgctggaaaacctgcaggcctaccagaaacggatgggcgtgcagatgcagcggttcaagtacccctacgacgtgcccgactacgcctgatgagcggccgcgagctc

SEQ ID NO: 41 - protein, 279 aa, synthetic construct
  REGION 1..279: note = Influenza H1N1&H5N1 M1 consensus sequence
MDWTWILFLVAAATRVHSMSLLTEVETYVLSIIPSGPLKAEIAQRLEDVFAGKNTDLEALMEWLKTRPILSPLTKGILGFVFTLTVPSERGLQRRRFVQNALNGNGDPNNMDRAVKLYKKLKREITFHGAKEVALSYSTGALASCMGLIYNRMGTVTTEVAFGLVCATCEQIADSQHRSHRQMATTTNPLIRHENRMVLASTTAKAMEQMAGSSEQAAEAMEVASQARQMVQAMRTIGTHPSSSAGLRDDLLENLQAYQKRMGVQMQRFKYPYDVPDYA

SEQ ID NO: 42 - DNA, 1700 bp, synthetic construct
  misc_feature 1..1700: note = Influenza H5N1 M2E-NP consensus sequence
  source 1..1700: mol_type = other DNA
ggtaccgaattcgccaccatggactggacctggatcctgttcctggtcgctgccgccaccagggtgcacagcagcctgctgaccgaggtggagacccccacccggaacgagtggggctgccggtgcagcgacagcagcgaccggggcaggaagcggagaagcgccagccagggcaccaagcggagctacgagcagatggaaacaggcggcgagcggcagaacgccaccgagatccgggccagcgtgggcagaatggtcggcggcatcggccggttctacatccagatgtgcaccgagctgaagctgtccgactacgagggccggctgatccagaacagcatcaccatcgagcggatggtgctgtccgccttcgacgagcggcggaacagatacctggaagagcaccccagcgccggcaaggaccccaagaaaaccggcggacccatctaccggcggagggacggcaagtgggtgcgggagctgatcctgtacgacaaagaggaaatccggcggatctggcggcaggccaacaacggcgaggacgccacagccggcctgacccacctgatgatctggcacagcaacctgaacgacgccacctaccagcggacaagggctctggtccggaccggcatggacccccggatgtgcagcctgatgcagggcagcacactgcccagaagaagcggagccgctggcgcagccgtgaagggcgtgggcaccatggtgatggaactgatccggatgatcaagcggggcatcaacgaccggaatttttggaggggcgagaacggcaggcggacccggatcgcctacgagcggatgtgcaacatcctgaagggcaagttccagacagccgcccagcgggccatgatggaccaggtccgggagagccggaaccccggcaacgccgagatcgaggacctgatcttcctggccagaagcgccctgatcctgcggggcagcgtggcccacaagagctgcctgcccgcctgcgtgtacggactggccgtggccagcggctacgacttcgagcgggagggctacagcctggtcggcatcgaccccttccggctgctgcagaactcccaggtgttcagcctgatccggcccaacgagaaccccgcccacaagtcccagctggtctggatggcctgccacagcgccgccttcgaggatctgagagtgagcagcttcatccggggcaccagagtggtgcccaggggccagctgtccaccaggggcgtgcagatcgccagcaacgagaacatggaagccatggacagcaacaccctggaactgcggagccggtactgggccatccggaccagaagcggcggcaacaccaaccagcagcgggccagcgccggacagatcagcgtgcagcccaccttctccgtgcagcggaacctgcccttcgagagggccaccatcatggccgccttcaccggcaacaccgagggccggaccagcgacatgcggaccgagatcatcaggatgatggaaagcgccaggcccgaggacgtgagcttccagggcaggggcgtgttcgagctgtccgatgagaaggccaccaaccccatcgtgcccagcttcgacatgaacaacgagggcagctacttcttcggcgacaacgccgaggaatacgacaactacccctacgacgtgcccgactacgcctgatgagcggccgcgagctc

SEQ ID NO: 43 - protein, 554 aa, synthetic construct
  REGION 1..554: note = Influenza H5N1 M2E-NP consensus sequence
MDWTWILFLVAAATRVHSSLLTEVETPTRNEWGCRCSDSSDRGRKRRSASQGTKRSYEQMETGGERQNATEIRASVGRMVGGIGRFYIQMCTELKLSDYEGRLIQNSITIERMVLSAFDERRNRYLEEHPSAGKDPKKTGGPIYRRRDGKWVRELILYDKEEIRRIWRQANNGEDATAGLTHLMIWHSNLNDATYQRTRALVRTGMDPRMCSLMQGSTLPRRSGAAGAAVKGVGTMVMELIRMIKRGINDRNFWRGENGRRTRIAYERMCNILKGKFQTAAQRAMMDQVRESRNPGNAEIEDLIFLARSALILRGSVAHKSCLPACVYGLAVASGYDFEREGYSLVGIDPFRLLQNSQVFSLIRPNENPAHKSQLVWMACHSAAFEDLRVSSFIRGTRVVPRGQLSTRGVQIASNENMEAMDSNTLELRSRYWAIRTRSGGNTNQQRASAGQISVQPTFSVQRNLPFERATIMAAFTGNTEGRTSDMRTEIIRMMESARPEDVSFQGRGVFELSDEKATNPIVPSFDMNNEGSYFFGDNAEEYDNYPYDVPDYA

SEQ ID NO: 44 - protein, 701 aa, Human immunodeficiency virus type 1
MDWTWILFLVAAATRVHSEEKLWVTVYYGVPVWKEATTTLFCASDAKAHHAEAHNVWATHACVPTDPNPQEVILENVTEKYNMWKNNMVDQMHEDIISLWDQSLKPCVKLTPLCVTLNCTNATYTNSDSKNSTSNSSLEDSGKGDMNCSFDVTTSIDKKKKTEYAIFDKLDVMNIGNGRYTLLNCNTSVITQACPKMSFEPIPIHYCTPAGYAILKCNDNKFNGTGPCTNVSTIQCTHGIKPVVSTQLLLNGSLAEGGEVIIRSENLTDNAKTIIVQLKEPVEINCTRPNNNTRKSIHMGPGAAFYARGEVIGDIRQAHCNISRGRWNDTLKQIAKKLREQFNKTISLNQSSGGDLEIVMHTFNCGGEFFYCNTTQLFNSTWNENDTTWNNTAGSNNNETITLPCRIKQIINRWQEVGKAMYAPPISGPINCLSNITGLLLTRDGGDNNNTIETFRPGGGDMRDNWRSELYKYKVVRIEPLGIAPTKAKRRVVQREKRAVGIGAMFLGFLGAAGSTMGAASVTLTVQARLLLSGIVQQQNNLLRAIEAQQHLLQLTVWGIKQLQARVLAMERYLKDQQLLGIWGCSGKLICTTNVPWNASWSNKSLDKIWHNMTWMEWDREIDNYTKLIYTLIEASQIQQEKNEQELLELDSWASLWSWFDISKWLWYIGVFIIVIGGLVGLKIVFAVLSIVNRVRQVTRV